European Patent Application EP 4 696 769 A1, published February 18, 2026. Title: METHOD FOR PRODUCING YEAST PRODUCT USING HIGH-LACTIC ACID INDUSTRIAL BY-PRODUCT. Applicant: ANGEL YEAST CO.,LTD. The sequence listing filed with the application follows.

SEQUENCE LISTING (4 sequences)

SEQ ID NO: 1 - DNA, 19 bp, synthetic construct
  source 1..19: mol_type = other DNA; note = synthetic DNA used as primer
tccgtaggtgaacctgcgg

SEQ ID NO: 2 - DNA, 20 bp, synthetic construct
  source 1..20: mol_type = other DNA; note = synthetic DNA used as primer
tcctccgcttattgatatgc

SEQ ID NO: 3 - DNA, 562 bp, Kluyveromyces marxianus
  source 1..562: mol_type = genomic DNA
ccaacggggattgccttagtacggcgagtgaagcggcaaaagctcaaatttgaaatctggcgtcttcgacgtccgagttgtaatttgaagaaggcgactttgtagctggtccttgtctatgttccttggaacaggacgtcatagagggtgagaatcccgtgtggcgaggatcccagttatttgtaaagtgctttcgacgagtcgagttgtttgggaatgcagctctaagtgggtggtaaattccatctaaagctaaatattggcgagagaccgatagcgaacaagtacagtgatggaaagatgaaaagaactttgaaaagagagtgaaaaagtacgtgaaattgttgaaagggaagggcatttgatcagacatggcgtttgcttcggctttcgctgggccagcatcagttttagcggttggataaatcctcgggaatgtggctctgcttcggtagagtgttatagcccgtgggaatacagccagctgggactgaggattgcgacttttgtcaaggatgctggcgtaatggttaaatgccgcccgtcttgaacccacggacca

SEQ ID NO: 4 - DNA, 716 bp, Kluyveromyces lactis
  source 1..716: mol_type = genomic DNA
tccggggaatctacctgatttgaggtcaactttgagagttttgattaagccgtatgcctcaaggagacaaacaccagcgagtctttataacacctataagctcattgaccctagcttaccacgaattggcgcaaacctaagacgtagatgtgcaagagtcgagtccatagacttgacacgcagccctgctcacgcagaaggcaacggctagccactttcaagttaacccgaaaaacgagtatcactcactaccaaacccaaaggtttgagagagaaatgacgctcaaacaggcatgccccctggaataccagagggcgcaatgtgcgttcaaagatttgatgattcacgaaaatctgcaattcacaatacatatcgcaattcgctgcgttcttcatcgatgcgagaaccaagagatccgttgttgaaagttttgaatattaaatttcttgataaatagtttttcataatgcaaaatgttgtttgtgtttatgtccactggagagacgagctctccagggaagtagttcatagagaaaaaactccattgtgtttaggatgagagaaagaaaactgatagcagaaaatcaagaattagccgcgcaattaagcgcaggccatattcagcgattcccccagtaatctactcattcataatctttaatgatccttccgcaggttcacctacggaaaccttgttacgattttttacctccaa